European Patent Specification EP 3 289 106 B1, published August 20, 2025. Title: Diagnostic Methods. Applicant: Griffith University. The sequence listing filed with the application follows.

SEQUENCE LISTING (64 sequences)

SEQ ID NO: 1 - DNA, 30 bp, Artificial Sequence
  Single stranded oligonucleotide
acgttggatgagcctccttctgacttgaac

SEQ ID NO: 2 - DNA, 30 bp, Artificial Sequence
  Oligonucleotide for detecting SNP
acgttggatgcatttcacctacaagtgatg

SEQ ID NO: 3 - DNA, 19 bp, Artificial Sequence
  Oligonucleotide for detecting SNP
cgatggaatttgacccaac

SEQ ID NO: 4 - DNA, 29 bp, Artificial Sequence
  Oligonucleotide for detecting SNP
acgttggatggctccgtatgtgctgagag

SEQ ID NO: 5 - DNA, 30 bp, Artificial Sequence
  Oligonucleotide for detecting SNP
acgttggatgagaaatacagcgctggcttc

SEQ ID NO: 6 - DNA, 16 bp, Artificial Sequence
  Oligonucleotide for detecting SNP
aggggcttgtgtgtaa

SEQ ID NO: 7 - DNA, 30 bp, Artificial Sequence
  Oligonucleotide for detecting SNP
acgttggatgttctcacagttaaggccttg

SEQ ID NO: 8 - DNA, 30 bp, Artificial Sequence
  Oligonucleotide for detecting SNP
acgttggatggctgctaatgatagaggctg

SEQ ID NO: 9 - DNA, 23 bp, Artificial Sequence
  Oligonucleotide for detecting SNP
tacatggggatttacatagacta

SEQ ID NO: 10 - DNA, 30 bp, Artificial Sequence; identical to SEQ ID NO: 7
  Oligonucleotide for detecting SNP

SEQ ID NO: 11 - DNA, 30 bp, Artificial Sequence; identical to SEQ ID NO: 8
  Oligonucleotide for detecting SNP

SEQ ID NO: 12 - DNA, 23 bp, Artificial Sequence
  Oligonucleotide for detecting SNP
tacatggggatttacatagacta

SEQ ID NO: 13 - DNA, 30 bp, Artificial Sequence; identical to SEQ ID NO: 7
  Oligonucleotide for detecting SNP

SEQ ID NO: 14 - DNA, 30 bp, Artificial Sequence; identical to SEQ ID NO: 8
  Oligonucleotide for detecting SNP

SEQ ID NO: 15 - DNA, 23 bp, Artificial Sequence
  Oligonucleotide for detecting SNP
tacatggggatttacatagacta

SEQ ID NO: 16 - DNA, 30 bp, Artificial Sequence
  Oligonucleotide for detecting SNP
acgttggatgctcaggcaaagggtattcac

SEQ ID NO: 17 - DNA, 30 bp, Artificial Sequence
  Oligonucleotide for detecting SNP
acgttggatgagaacctaagaacccaaggc

SEQ ID NO: 18 - DNA, 24 bp, Artificial Sequence
  Oligonucleotide for detecting SNP
gggaagagatttagaggttgtacc

SEQ ID NO: 19 - DNA, 30 bp, Artificial Sequence
  Oligonucleotide for detecting SNP
acgttggatgttgctggtggtggcttaaac

SEQ ID NO: 20 - DNA, 30 bp, Artificial Sequence
  Oligonucleotide for detecting SNP
acgttggatgctagggtgaacaacttgaac

SEQ ID NO: 21 - DNA, 24 bp, Artificial Sequence
  Oligonucleotide for detecting SNP
ggggacctttcaaaagagtgatac

SEQ ID NO: 22 - DNA, 30 bp, Artificial Sequence
  Oligonucleotide for detecting SNP
acgttggatgaaggttcaagttgttcaccc

SEQ ID NO: 23 - DNA, 30 bp, Artificial Sequence
  Oligonucleotide for detecting SNP
acgttggatgttacctgccttttaccacac

SEQ ID NO: 24 - DNA, 20 bp, Artificial Sequence
  Oligonucleotide for detecting SNP
ccctccttccaggaacttac

SEQ ID NO: 25 - DNA, 30 bp, Artificial Sequence
  Oligonucleotide for detecting SNP
acgttggatgagtgttccaatcgctctgtg

SEQ ID NO: 26 - DNA, 29 bp, Artificial Sequence
  Oligonucleotide for detecting SNP
acgttggatgaatcaactgagaaccattc

SEQ ID NO: 27 - DNA, 26 bp, Artificial Sequence
  Oligonucleotide for detecting SNP
cttctaatatacagccatgtcataga

SEQ ID NO: 28 - DNA, 30 bp, Artificial Sequence
  Oligonucleotide for detecting SNP
acgttggatgggaaaaacaatttcttgggg

SEQ ID NO: 29 - DNA, 30 bp, Artificial Sequence
  Oligonucleotide for detecting SNP
acgttggatgcccacctatgaccattttcc

SEQ ID NO: 30 - DNA, 18 bp, Artificial Sequence
  Oligonucleotide for detecting SNP
gaccattttcctcagaga

SEQ ID NO: 31 - DNA, 29 bp, Artificial Sequence
  Oligonucleotide for detecting SNP
acgttggatgcatcaagacagatttcaac

SEQ ID NO: 32 - DNA, 30 bp, Artificial Sequence
  Oligonucleotide for detecting SNP
acgttggatgcctacatctcatcaaaggac

SEQ ID NO: 33 - DNA, 27 bp, Artificial Sequence
  Oligonucleotide for detecting SNP
ggtacagaataagaaagtttgagatta

SEQ ID NO: 34 - DNA, 30 bp, Artificial Sequence
  Oligonucleotide for detecting SNP
acgttggatgcgtttgtgtttatgcccctc

SEQ ID NO: 35 - DNA, 31 bp, Artificial Sequence
  Oligonucleotide for detecting SNP
acgttggatgggagtttgctatattattccc

SEQ ID NO: 36 - DNA, 25 bp, Artificial Sequence
  Oligonucleotide for detecting SNP
ggggcaccattacaggtaatttcca

SEQ ID NO: 37 - DNA, 30 bp, Artificial Sequence
  Oligonucleotide for detecting SNP
acgttggatgttttcccttattcctcccac

SEQ ID NO: 38 - DNA, 30 bp, Artificial Sequence
  Oligonucleotide for detecting SNP
acgttggatgacctctagcctctgaattgc

SEQ ID NO: 39 - DNA, 20 bp, Artificial Sequence
  Oligonucleotide for detecting SNP
ggaggagaaacaaactccag

SEQ ID NO: 40 - DNA, 29 bp, Artificial Sequence
  Oligonucleotide for detecting SNP
acgttggatgaaagtgggcggggacatag

SEQ ID NO: 41 - DNA, 30 bp, Artificial Sequence
  Oligonucleotide for detecting SNP
acgttggatgaaaaacacgccccattgctc

SEQ ID NO: 42 - DNA, 15 bp, Artificial Sequence
  Oligonucleotide for detecting SNP
aagtcacgccccttc

SEQ ID NO: 43 - DNA, 30 bp, Artificial Sequence
  Oligonucleotide for detecting SNP
acgttggatggaaatgatgctttccacggg

SEQ ID NO: 44 - DNA, 30 bp, Artificial Sequence
  Oligonucleotide for detecting SNP
acgttggatgaactgcctgagcctacagac

SEQ ID NO: 45 - DNA, 26 bp, Artificial Sequence
  Oligonucleotide for detecting SNP
ctgcatgagcctacagaccaccttct

SEQ ID NO: 46 - DNA, 30 bp, Artificial Sequence
  Oligonucleotide for detecting SNP
acgttggatggaggcttttaatcaactccc

SEQ ID NO: 47 - DNA, 31 bp, Artificial Sequence
  Oligonucleotide for detecting SNP
acgttggatggataatttttctgtgacagac

SEQ ID NO: 48 - DNA, 24 bp, Artificial Sequence
  Oligonucleotide for detecting SNP
gacactgtctttcatttgacttgt

SEQ ID NO: 49 - DNA, 30 bp, Artificial Sequence
  Oligonucleotide for detecting SNP
acgttggatgctggtgggagaatgcaagtc

SEQ ID NO: 50 - DNA, 30 bp, Artificial Sequence
  Oligonucleotide for detecting SNP
acgttggatgggctaatagtcccttttacc

SEQ ID NO: 51 - DNA, 23 bp, Artificial Sequence
  Oligonucleotide for detecting SNP
ggggtcatgtttttccattgtca

SEQ ID NO: 52 - DNA, 30 bp, Artificial Sequence
  Oligonucleotide for detecting SNP
acgttggatgtgtcaacctagtagacgagc

SEQ ID NO: 53 - DNA, 30 bp, Artificial Sequence
  Oligonucleotide for detecting SNP
acgttggatgtggagatgcatcctctaggc

SEQ ID NO: 54 - DNA, 17 bp, Artificial Sequence
  Oligonucleotide for detecting SNP
aggcgaaagctctaatt

SEQ ID NO: 55 - DNA, 30 bp, Artificial Sequence
  Oligonucleotide for detecting SNP
acgttggatgaccatctgcaggactttagg

SEQ ID NO: 56 - DNA, 30 bp, Artificial Sequence
  Oligonucleotide for detecting SNP
acgttggatgcttttggggctgagtttaag

SEQ ID NO: 57 - DNA, 27 bp, Artificial Sequence
  Oligonucleotide for detecting SNP
ccccgctcttccttcaaaactatcttg

SEQ ID NO: 58 - DNA, 30 bp, Artificial Sequence
  Oligonucleotide for detecting SNP
acgttggatggggtaaaagaattacacaag

SEQ ID NO: 59 - DNA, 29 bp, Artificial Sequence
  Oligonucleotide for detecting SNP
acgttggatgtgcctgaattatgcaatag

SEQ ID NO: 60 - DNA, 21 bp, Artificial Sequence
  Oligonucleotide for detecting SNP
tatgcaatagaatcacttggt

SEQ ID NO: 61 - DNA, 30 bp, Artificial Sequence
  Oligonucleotide for detecting SNP
acgttggatgtcttctccagtgtctaaggg

SEQ ID NO: 62 - DNA, 30 bp, Artificial Sequence
  Oligonucleotide for detecting SNP
acgttggatgcccaatgttacatggcttcc

SEQ ID NO: 63 - DNA, 15 bp, Artificial Sequence
  Oligonucleotide for detecting SNP
aggctacagagctga

SEQ ID NO: 64 - DNA, 50 bp, Artificial Sequence
  Single standed polynucleotide
ctcatcctgtctttgcaggagattctgggtatatagttcctccagagaca